European Patent Specification EP 3 929 205 B1, published April 8, 2026. Title: Method of producing complementary modified oligonucleotide. Applicant: Ajinomoto Co., Inc. The sequence listing filed with the application follows.

SEQUENCE LISTING (82 sequences)

SEQ ID NO: 1 - RNA, 21 nt, Artificial Sequence
  oligonucleotide
aacaguguucuugcucuauaa

SEQ ID NO: 2 - RNA, 23 nt, Artificial Sequence
  oligonucleotide
uuauagagcaagaacacuguuuu

SEQ ID NO: 3 - RNA, 12 nt, Artificial Sequence
  oligonucleotide
cuugcucuauaa

SEQ ID NO: 4 - RNA, 10 nt, Artificial Sequence
  oligonucleotide
aacaguguuc

SEQ ID NO: 5 - RNA, 11 nt, Artificial Sequence
  oligonucleotide
uugcucuauaa

SEQ ID NO: 6 - RNA, 11 nt, Artificial Sequence
  oligonucleotide
aacaguguucu

SEQ ID NO: 7 - RNA, 10 nt, Artificial Sequence
  oligonucleotide
ugcucuauaa

SEQ ID NO: 8 - RNA, 12 nt, Artificial Sequence
  oligonucleotide
aacaguguucuu

SEQ ID NO: 9 - RNA, 10 nt, Artificial Sequence
  oligonucleotide
uuauagagca

SEQ ID NO: 10 - RNA, 13 nt, Artificial Sequence
  oligonucleotide
agaacacuguuuu

SEQ ID NO: 11 - RNA, 11 nt, Artificial Sequence
  oligonucleotide
uuauagagcaa

SEQ ID NO: 12 - RNA, 12 nt, Artificial Sequence
  oligonucleotide
gaacacuguuuu

SEQ ID NO: 13 - RNA, 12 nt, Artificial Sequence
  oligonucleotide
uuauagagcaag

SEQ ID NO: 14 - RNA, 11 nt, Artificial Sequence
  oligonucleotide
aacacuguuuu

SEQ ID NO: 15 - RNA, 13 nt, Artificial Sequence
  oligonucleotide
uuauagagcaaga

SEQ ID NO: 16 - RNA, 10 nt, Artificial Sequence
  oligonucleotide
acacuguuuu

SEQ ID NO: 17 - protein, 342 aa, Deinococcus radiodurans
MAERQVIKERAQLFPHPNAERLELCKVGTFQLVVRKGEYRDGDPIVIAPEKAVLPPQLAGLYTNADTGASYLHGAEKNRVGSVRLRGEVSQGVILPLDGLEDAPFGEDLAERLGITFWEPPVPVSMAGEVEPRPPAQHYKHHDVEQFGIYVSEFASGEEVMVTEKLHGTQGVYFRTAEGRWLVTSKGLSRGGLTLREAASNVYWQAARNSNLFAEADAAFSGGEVQIFGEVVPVQKGFSYGQHKPTVFVFKVVYDGLRLPRRDWPQWVLDHAVPVLYEGPFDEATVRKLRGGLETVSGKGLHIREGVVVAPKVPRFAADGSDLSVKLISDAYAKKETGEEYS

SEQ ID NO: 18 - DNA, 51 bp, Artificial Sequence
  oligonucleotide
caugagugacaaagcauucccaacggaaugcuuugucacucauggcutcgg

SEQ ID NO: 19 - DNA, 12 bp, Artificial Sequence
  oligonucleotide
caugagugacaa

SEQ ID NO: 20 - DNA, 15 bp, Artificial Sequence
  oligonucleotide
agcauucccaacgga

SEQ ID NO: 21 - DNA, 11 bp, Artificial Sequence
  oligonucleotide
augcuuuguca

SEQ ID NO: 22 - DNA, 13 bp, Artificial Sequence
  oligonucleotide
cucauggcutcgg

SEQ ID NO: 23 - DNA, 13 bp, Artificial Sequence
  oligonucleotide
gcactggcagtcg

SEQ ID NO: 24 - DNA, 13 bp, Artificial Sequence
  oligonucleotide
cgacugccagugc

SEQ ID NO: 25 - RNA, 21 nt, Artificial Sequence
  oligonucleotide
aacgguguucuugcucuauaa

SEQ ID NO: 26 - RNA, 23 nt, Artificial Sequence
  oligonucleotide
uuauagagcaagaacacuguuuu

SEQ ID NO: 27 - RNA, 12 nt, Artificial Sequence
  oligonucleotide
aacgguguucuu

SEQ ID NO: 28 - RNA, 13 nt, Artificial Sequence
  oligonucleotide
uuauagagcaaga

SEQ ID NO: 29 - RNA, 10 nt, Artificial Sequence
  oligonucleotide
acacuguuuu

SEQ ID NO: 30 - RNA, 21 nt, Artificial Sequence
  oligonucleotide
ccgcuagggugagcauagcug

SEQ ID NO: 31 - RNA, 21 nt, Artificial Sequence
  oligonucleotide
cagcuaugcucacccuagcgg

SEQ ID NO: 32 - RNA, 12 nt, Artificial Sequence
  oligonucleotide
ugagcauagcug

SEQ ID NO: 33 - DNA, 21 bp, Artificial Sequence
  oligonucleotide
guaaccaagaguauuccautt

SEQ ID NO: 34 - DNA, 21 bp, Artificial Sequence
  oligonucleotide
auggaauacucuugguuactt

SEQ ID NO: 35 - RNA, 11 nt, Artificial Sequence
  oligonucleotide
guaaccaagag

SEQ ID NO: 36 - DNA, 10 bp, Artificial Sequence
  oligonucleotide
uauuccautt

SEQ ID NO: 37 - RNA, 12 nt, Artificial Sequence
  oligonucleotide
auggaauacucu

SEQ ID NO: 38 - RNA, 53 nt, Artificial Sequence
  oligonucleotide
  misc_feature (25)..(25): proline residue
  misc_feature (52)..(52): proline residue
agcagaguacacacagcauauaccngguauaugcuguguguacucugcuucng

SEQ ID NO: 39 - RNA, 14 nt, Artificial Sequence
  oligonucleotide
agcagaguacacac

SEQ ID NO: 40 - RNA, 15 nt, Artificial Sequence
  oligonucleotide
  misc_feature (11)..(11): proline residue
agcauauaccnggua

SEQ ID NO: 41 - RNA, 12 nt, Artificial Sequence
  oligonucleotide
uaugcugugugu

SEQ ID NO: 42 - RNA, 12 nt, Artificial Sequence
  oligonucleotide
  misc_feature (11)..(11): proline residue
acucugcuucng

SEQ ID NO: 43 - RNA, 21 nt, Artificial Sequence
  oligonucleotide
gcuaaccggggggggugccag

SEQ ID NO: 44 - RNA, 21 nt, Artificial Sequence
  oligonucleotide
cuggcaccccccccgguuagc

SEQ ID NO: 45 - RNA, 14 nt, Artificial Sequence
  oligonucleotide
gcuaaccggggggg

SEQ ID NO: 46 - RNA, 13 nt, Artificial Sequence
  oligonucleotide
gcuaaccgggggg

SEQ ID NO: 47 - RNA, 12 nt, Artificial Sequence
  oligonucleotide
gcuaaccggggg

SEQ ID NO: 48 - RNA, 11 nt, Artificial Sequence
  oligonucleotide
gcuaaccgggg

SEQ ID NO: 49 - RNA, 10 nt, Artificial Sequence
  oligonucleotide
ggggugccag

SEQ ID NO: 50 - RNA, 10 nt, Artificial Sequence
  oligonucleotide
gcuaaccggg

SEQ ID NO: 51 - RNA, 11 nt, Artificial Sequence
  oligonucleotide
gggggugccag

SEQ ID NO: 52 - RNA, 12 nt, Artificial Sequence
  oligonucleotide
ggggggugccag

SEQ ID NO: 53 - RNA, 13 nt, Artificial Sequence
  oligonucleotide
cuggcaccccccc

SEQ ID NO: 54 - RNA, 14 nt, Artificial Sequence
  oligonucleotide
gcccacgauagugc

SEQ ID NO: 55 - RNA, 14 nt, Artificial Sequence
  oligonucleotide
gcacuaucgugggc

SEQ ID NO: 56 - RNA, 13 nt, Artificial Sequence
  oligonucleotide
gcccacgaugugc

SEQ ID NO: 57 - RNA, 13 nt, Artificial Sequence
  oligonucleotide
gcacaucgugggc

SEQ ID NO: 58 - RNA, 12 nt, Artificial Sequence
  oligonucleotide
gcccacgugugc

SEQ ID NO: 59 - RNA, 12 nt, Artificial Sequence
  oligonucleotide
gcacacgugggc

SEQ ID NO: 60 - RNA, 11 nt, Artificial Sequence
  oligonucleotide
gcccacgugug

SEQ ID NO: 61 - RNA, 11 nt, Artificial Sequence
  oligonuleotide
cacacgugggc

SEQ ID NO: 62 - DNA, 28 bp, Artificial Sequence
  oligonucleotide
gggtaatgaattccaaagcttcccccta

SEQ ID NO: 63 - DNA, 28 bp, Artificial Sequence
  oligonucleotide
tagggggaagctttggaattcattaccc

SEQ ID NO: 64 - DNA, 19 bp, Artificial Sequence
  oligonucleotide
attccaaagcttcccccta

SEQ ID NO: 65 - DNA, 16 bp, Artificial Sequence
  oligonucleotide
tagggggaagctttgg

SEQ ID NO: 66 - DNA, 12 bp, Artificial Sequence
  oligonucleotide
aattcattaccc

SEQ ID NO: 67 - RNA, 28 nt, Artificial Sequence
  oligonucleotide
ggguaaugaauuccaaagcuucccccua

SEQ ID NO: 68 - RNA, 28 nt, Artificial Sequence
  oligonucleotide
uagggggaagcuuuggaauucauuaccc

SEQ ID NO: 69 - RNA, 19 nt, Artificial Sequence
  oligonucleotide
auuccaaagcuucccccua

SEQ ID NO: 70 - RNA, 16 nt, Artificial Sequence
  oligonucleotide
uagggggaagcuuugg

SEQ ID NO: 71 - RNA, 12 nt, Artificial Sequence
  oligonucleotide
aauucauuaccc

SEQ ID NO: 72 - RNA, 25 nt, Artificial Sequence
  oligonucleotide
ggguaaugaauuccaaagcuucccc

SEQ ID NO: 73 - RNA, 29 nt, Artificial Sequence
  oligonucleotide
ggggaagcuuugguagggggaagcuuugg

SEQ ID NO: 74 - RNA, 16 nt, Artificial Sequence
  oligonucleotide
auuccaaagcuucccc

SEQ ID NO: 75 - RNA, 13 nt, Artificial Sequence
  oligonucleotide
ggggaagcuuugg

SEQ ID NO: 76 - RNA, 23 nt, Artificial Sequence
  oligonucleotide
ggguaaugaauuccaaagcuucc

SEQ ID NO: 77 - RNA, 27 nt, Artificial Sequence
  oligonucleotide
ggaagcuuugguagggggaagcuuugg

SEQ ID NO: 78 - RNA, 14 nt, Artificial Sequence
  oligonucleotide
auuccaaagcuucc

SEQ ID NO: 79 - RNA, 11 nt, Artificial Sequence
  oligonucleotide
ggaagcuuugg

SEQ ID NO: 80 - RNA, 21 nt, Artificial Sequence
  oligonucleotide
ggguaaugaauuccaaagcuu

SEQ ID NO: 81 - RNA, 21 nt, Artificial Sequence
  oligonucleotide
aagcuuuggaauucauuaccc

SEQ ID NO: 82 - RNA, 12 nt, Artificial Sequence
  oligonucleotide
auuccaaagcuu